European Patent Specification EP 3 483 283 B1, published August 27, 2025. Title: Method of screening for a prophylactic or therapeutic agent for diseases caused by Interleukin 6 or CXCL5. Applicant: THE UNIVERSITY OF TOKYO TAK-Circulator Corporation. The sequence listing filed with the application follows.

SEQUENCE LISTING (28 sequences)

SEQ ID NO: 1 - DNA, 3532 bp, Human
tcaagaggcggggaggagaggaggaaaaagcgctgagtgagggcgggcgggcgggcgggagggagggagtggaggagccggggaggggctccttaaagaaacgcttctgtcgctcgcctgctcgcttttcgctcggcattgcggccagccagccgggcactcggggggcacgcgcggccaccgctagagctctgcccccaccccacccgccagcaggtctggggtggggacccaggtgggggctcctgcagccactgcccggtgcggaccgcacggagcgacccactcctcccagcaccgaggaagaagcaacggagccctcagcaggcgaccggcctccccgcccctgaccacccgcttcccggctgcctttgtggccgcagcttctcgccgccgagccgagggccggcgggggcgcggcgcgcacggccgagcgatgcccagctcgctgttcgcagacctggagcgcaacggcagcggcggcggcggcggcggcagcagcggagggggagagaccctggatgaccaaagagccctgcagctcgcgctcgaccagctctccctgctggggctggacagtgacgagggcgcctctctgtacgacagcgagccgcgcaagaagagcgtgaacatgaccgagtgcgtgccagtacccagttctgagcatgtcgccgagatcgtggggcggcaaggttgtaaaatcaaagcgctgcgggcgaagaccaatacttacatcaagaccccagttcgcggggaggagcctgtctttgttgtgacgggcaggaaggaggatgtggccatggctcggagggagatcatctctgctgccgagcacttctccatgatccgcgcctcccggaataagaacacggcactcaacggcgcggtgcctgggccgcccaacctgcccgggcagaccaccatccaagtgcgggtaccctaccgcgtggtggggctcgtggtggggcccaaaggcgccacaatcaagcgcatccagcagcagacgcacacgtacatcgtgacgcccagccgggataaggagccggtgttcgaggtgaccggcatgccagagaacgtggatcgcgctcgagaggagattgaggcgcacattgctctgcgtaccggcggcatcattgagctcacagacgagaacgacttccacgccaacggcaccgatgtgggcttcgatctgcatcatgggtccggcgggtccggcccaggcagcctctggagcaagcccacccccagcatcacgcccacccccggccgcaagcctttctctagctaccgcaacgacagctccagctcgcttggcagtgcttccacagactcttatttcggcggcgggaccagcagcagcgcagcggctacccagcgcctggcggactacagcccccctagccccgccctgagctttgcgcacaacggaaacaataacaataacggcaatgggtacacctacacagcggggggagaagcctcagtgccatcccccgacggctgccccgagctgcagcccacttttgacccggctcccgctcccccacctggggcaccacttatctgggcccagttcgagcggtccccgggaggcggacctgcagctccggtatcttcttcctgctcttcttctgcatcttcgtctgcttcttcctcctccgtggtcttccccgggggtggcgccagtgcgccctccaacgccaacctggggctattggtgcaccgccggctgcaccctggcaccagctgcccgcgcctgtctccacccttgcacatggccccgggggcgggagagcaccacctggctcgccgggtgcgcagcgacccgggtggaggaggcctggcctacgccgcttatgccaacgggctgggggcacagctgcctggcttgcagccgtcggacacgtcgggctcctcctcttcgtccagctcctcctccagctcttcatcctcttcctccgggcttcggcgtaaaggcagccgcgactgctccgtgtgcttcgagagcgaagtgattgccgcgctggtgccctgtggccacaacctcttctgcatggagtgcgccaatcgcatctgtgagaagagcgagcccgagtgcccggtctgccacaccgcggtcactcaggccatccgcatcttttcttaaaggcagcgggcgctgctagtgcgcaccgtgctgggggaagggggaacccctccccatcctctttccccagcgctcgcctgcctccctgggtgccccccctctcccttctccttcccggccccaccaacactctgagatccgagaggagcttggaaagctgtagtatccgctcatttttaaaatttaatttttaagtaaaggaatttgccaggatatctgcatcaagagtactgtagcctgggaaacctgaacacctgaaatgcatgctctataaataataggaacggcgacattctagtaatgatagtttttacactgtacttaataggaagcttccaaaagaagaaaaccccacaagttttccattttcttaaagtaggaaaaaatgaacagtaataattatgatgaagatgatagtagtgctatgggatgtgtggactgtttagtgtgttcccctttgtgggtgggttcctatgatacttattatagaacacagtggatcctttttgaatgttcgtggaagggccaggagttcctgtgaaaccaggatactgcagctttattaaagttaaagaaactgtaacatatctcttatatattaaaaacgtttaaaagttttaaagagaaattgcattaatacagattgaagtattttattcttttttgacttgaaaaattatatttcatattgcaaagatgtttacaagtattttaatttaagttcagtgaacttttttgtagctgggttaaatctttttattttagtatggccttatggcaaagaacactgtattattttaataatcacacaattgtgacggaattacaaccataaaatgtgtaatgttttgaacagtattctgttgggatggagattttataggttcagacaaatcttctagatctgcttcacccagcatattttctattcagtgatataaagcatattttattctatattattacaaaaacggaaatgtataaacatgtcaaaaagaactgttgatgctttctaacatttgtataaatagaattcagtgcaagttacaaaaattctgttgcaccactctagttttagtatttctattttaatacatttgtttaccacttgtttatgtatatgtaggtgatgttacttgagcttaaatgtactttactgagcaaagtttaaaaaacaaagtatattttattttatgataaagggcctttaacctcatggtcaaatactaatattatatttgctgagacaagatttgaaattgtatcaagagttttatttttctgacatttaaagttctacataataaaggtaaaacttaagtaatggtgctacttcattttttaagtatttctatataaataaaatattgaagaaaatcttaaaaa

SEQ ID NO: 2 - DNA, 35919 bp, Human
ctccaggtgtgttactgaataacaacaacaataatggaatagtttgaaatgccaggcacagtctgaagtgtgttatagacttgtattatctcactcaagcctcacagcatccctgcgtgaaggtggaatcattatcccaaatttgcagacaagactgaggctcagagagatcagtaagtagtagagctgagattcaagcctggattcgcttgactccgtagtccatgtactaactaaccactaggttaaactcccttgttgggcctgacccatgaattggaaaaccagaacctggccccatcttcgtcagtacttggctgggtcaccttgagaaagtcactttccctctcctgtcctctgatttattatgagtcaaatacaggtagtacctatcagggtttcctgaagaggtacctatgaaaatgatttgtttccctgctgtaagtgataagaaaacctccaaagataatgcccccctgtctttttaaggcttctcattctttcttatggcactttctgctcatgagtggaaacttatgtgtatttactgcagggacaaccacattttgtccgcagagctatggggtgcagcaaaggaaggtaggatttggtacatttccccaactctctcctgaccagatccatatattctcagctggttggaggcgtgactccaatctaactgacccacaaaacctctgcctctctcccttctctgcttgactcatccattcttcagaacccagtttgggagatctcttccagaaaggcttctgtgaccatcagtctgagtgtggggcttctccttgagctcccaccaagctctctctcttttttttttcttttttccacacaggattgtgctctgtcactcaggctggagtccagtggtgcgatcatagctcactgcagccttgatctcctgggctgaagtgatctttccacctcagcctcccaagcagttgggaccacaggcatgcatcatcacgcctggctaattaaaaattttttttttcagagaaggggtcttgctatgttgtccaggctggtcttaaactcctgggctcaagcgatcctcccgccttggcctcccctagtactggggttacaggcatgagggactgagctgggcaccacgctctccttgtaacttcttcctctctccacaaaggcagggactttgattgtctaatgcctgatctgctgcccagcaggaacgctctcagtaaaagatgaatgaatgaaaaatgggtcagatgcacctgcaatgatgtgtgattcattctcaaagttgtgtgggtgtctggttggactctgctcatgttcctcctgtgtccccaggtcccacttctcactgatgcgccccaggcagtctgtggtgctctactctttctccagggccacctatcactgaacctacaggatggccctgatgaatcaggggcaggtggcacaggtggatggcaggggtacaatgtgccagaagtgaggtgttcaccccctgttcaggtggtttgggttggagtctaagctggtttcctctattcctgtcttactcaagggaaattcctacccctggccaagacagaaataggagaaaccagcttaaaatccatccctttcctctgagacagaaaaccatcaaagtgtaacacattcaccttatctaaggaaacctcaaatttactcaaaatggcagagagagaaaaatgcgtctcttgtgtgtgtggagttggagccacataatgcacattcagagggtttacacccctcatggaggattcttctccttataaagttgccacaaaagaagagacacagccatggatgctcacaacctaactaagattaggataagcctatggggcggggcggtggggcagacagacaggaatacaatgccttctgcctctgcatgccatttgtctttcagggaaatctggctgagaactgctgtagatacttgctatcagcaagacactctcccatttcctaccccagagttatgaggagtgtacgtgctgctggatgggagcagcgcctgggcagattccatagacagaaatgtgattctgatggaaataaaacaaacaaacaaagcaaactcagcaaaagtctcagcagtcatgaaccttctgggaaagagctgcactaaattaccgagtctcttcatttagatgaaagtgcgtgtcttgagacatcattgttattttaaccatctgggaggaaagtattctccctaaagcctgagctccttgaaggcagagctgtgtcttacataactctacatcatccatggcgcctggttgtagtagttgccttcccaatacctcttcttttcttctttaccaacagaacctctgtattgttggggtttgaagtaataagctacatttcccattcttcttgcacagagagatggcaaatgagatgtaagcaaaattgattaaagcgctgttagagctgtttgaaagggattgagaagaatgcctttttgctgtttccctttcctcctgcctgctgactggaatttacatgtgatgacttgtatttcagcagccattttgtgattatgagttgactttgaagatgaaagccacatgctataagaatggtgaagcaaaaagataggtttctaaagcttctgaacagcaaaggaaacaatcaaatgtaccccataaatatatacacctattatatgcccataataattaaaaaattaaaaaggggctgggagcagtggctcagacctataatcccagcactttgggaggccaaggcaggtggactgctgagctcgggagtttgagatcagcctgggcaacacggtgaaaccctgtctctaaaaaaaaaaaaaaaaaaaaaaattagctgggagtggtgtgtgcctgtgttcccagctactcaggaggctgaggtgggaggattgcttgagcccaggaggttgaggctgcagtgagccatgataacgttactgcactccagcctgggcctgttatgcaaaagtgcatgggctctgggagagaggttgggaggctcgcctttgaatatgggtattaagcttcagtggatgaattatatatcatttattaatatcttggctgctcagaaacctttttactcacttgcagctttggccacatcttaaacagctgcatagctagctctaaacaggtgagaattctgaacactacatctcaaatttcctttttttttttttttgagacagattcagattcttgctctgtcacccaggctggggtgcagtggcacggtcttggctccctgcaacctccgcctcccgggttcaagcgattctcctgcctcagcctccccagtagctaggattacaggcgcatgccaccacgctcggctacttttggtatttttagcagagacggtgtttcactatgttggccaggctggtctggaactcctggccttgtgatctgcccacctcggcctcccaaagtgctgggattacaggtgtgacccaccacgcccagccacatttcaaatttctaagagctcaggcacagggaggtgagcatgacatcaggtaagggaagtaagggttcggtctgtcgttcctgctggacactgaaggtggacgtgtatttgatgaccagatagaagatgggtccttgtgtagtcttttcacttcagaggagttcctttgctctcttggggcttcgggttccctttccatccagatgcccagatgctcctagactggttcttccctttcttccctggctttctgttttctgtgcttgctcaggggaatagtgtgggaagacagtttccctcacaggttcaaggcggtagagcgttgttgagggtctcctgctggagaagtggaactttgcgactgtcactcaggagtgcaatgcagtttctgagatgaaaatttgcgaaccaatttcacgtggtcaatgttgtgaatgaatttatagctagtgaggctctgagtgctgatcagctgggatgactttggagctagatctgaatactaatgggactgggtgactttagttggtgagaattttgagaccctctttgttttgtttaaaatggtctgaggcttttttttttttttttttttttttgagatggagtcttgctctgtcgcccaggctagagtcagtggtgtgatctcggcttaccgcaacctccgcctcccaggttcaagcgattctcctgcctcagcctgctgagtagctgggactacaggcgcctgccaccacgcccaggcaatttttggatttttagcagagacggtgtttcaccatgatggccaggctggtctggaactcctgaccttgtgatctgcccacctcggcctcccaaagtgctgagattacagccatgtgccaccacacccaggcgtattatatcaataacaatttcttagttttgacaaatgtaccatgattgtgtaagatgttactagtaggcaatgctggataaagggtatacaagaatcatatatgccatctttgtaactcttctgtaaatctaaaattattccaaaattaaaagtttaaaataatttttaaaaagtcaatcaccaaaaagtaagtacatttaggacatagatacatgcaagacatgtgtaacataactgaaaatcacagattttggagtcggacgtacctggtttctcatcctggctgccccaattgctaactgcaatgttgggcaaatttctttattccttcaagctctgtgttccaatctctaaaataggaatcctaattatatatacttcaaggggttcctgggaagagtaaatgagaaaatactggcaaagtgccttatcatagtgcctgattgcctgatacatagtaagagctcaataaaagtagcttttattattcttgcaggtgatcaaagaaatgcagagtcaaacaatgttggcaaatgatttcacacctactgaatcggcaacaactgtgatccccagtgcctgacagagtgtgctgaaaccggtacattcataaactgtaaaccagtacagctatttggaaaagcaacgtagcaatatagacacagcaagagactgcagaaatggtcacaacctttcgcccagacctcctcttaatgatttgcagggttccaggcaagggtataaatggagcctcacataccatatgtataagtagtttaaagttagaaatcaggttacaaactgttaaatgaaaatatgttctagcctcctgccttggcaaatatactgtcaccaccacctggaagggctcaagttaaaaattctcagatgcctctgcatcctgtgttggaacatgacggcatggggagagccagttgctagcccccagacccactgtctttccaattcctaagtctgtccagcactgagggggcctcatgtgaatgtgagtggacagcctagcccatgcgtccaaactctgttcactaccccctgcctgtggccactcctcagatccgggtgtgtctactggtggtgtgattggatctcaggaggagagactcagggaccagggctgggcaggccctggagatgagcatggggccagtgggcagggacttctgggagtcctaggcacctggagaatggtctaaaagggaggacgtggatttgcaatgggcatgttcccttggcctgcagactcctcaccaggtgggagggacgcagcccaaggagggccagggggacaccccctgcctgatctcactgcagtactccttagagtccatccaaaggaaagaaatagttcagcagaataaaaaggctacgggcacaaagatagtatcactgtgttgcatttgacactaaaaaaacccaatctaatgttcaacagtagggaaatgttaagacaacaatgataaagctattcagagaagtagtatgctaccaccaacactggcacatgtgacaaccatgtcataacatgggataatgtttatgtgtagatataatagtaaatgaactctggcaactgtgcaaacatctgtgcgccctaggtgagatgcggaagtcaacctgcagacatgagaacagctgcctcaaagagggttgaactctttcaggcagctgaaagattttcctcccaaaattgtctctttcctgtggctggggagaagcagggacttttcaggaactaatgggtaagagctggctggttagactggagttttttgtgcaactctactcaggagttggagataagaacctgctacctgctgcatggaagccagaaaagcactttagctaatcacactccctctctgcgtgggctgaagatatccttgagtcctcccagccctgagcccttctccaggggccagcacacccagaaaccacgcgtgcagtgtttgctctggatgcccaggatagtctctgctgcgcgtgtgaagctctgccatgggctgggtatggaacgggccatgtcacactgagtcctcgcaacaacctggtgagatgggagcctcagcatggctgacttggacactgagatgctggtccagcaccacgcagttggcaagcagagaagccagcctttgaaactctgtgcttccatttgggcacgtacactgggaaatcaaaaggcagtgttccctttctccccacaaactgcttctagtgtcccatggggccagaggaactcaatcaaaacaatattccatagatgtgggatagtggtagcacaaataaattaacaattgcacttctgggcactcgactgtccccacggttctaaaaatgaaaagactctggtatttaatttatattttataagagtgaaaaaggccaggcacagtagctcacacctttaatcccatcattttggaaggccaaggtgggaggattgcttgaactcaagagttcaagaccagcctgggcaatatggcaaaactctacaaaaaaattagccgggtgtggtggtgcatgcctatagttccagctactcagagactgaggtgggaggatcacttgagcctgggaggtcgagactgcagtgcgccaagatagcaccactgtacttcagcctgggaaacagtgagattctgtctcaaaaaaaaaaaaaaaaaaaaaaaaatttgataattgcctttggtaaggaagagctgattttagcatggaacagagggtggcaaacaacagccttcaagccaaatctattccactgcttgtttttatatgtcccatgatctaaataatgggttttacatttttaaatggttggtggggggaaatgtgaaacttacatgaaattccagtctccagatctataaataaagttttattggaacacagccacattcagttgtgcatatgtattgtctacggcagcttctgcactataccagcagagttgaggagttgtaacagggagatcatatggcctgaaaagctgaaaaattttactatctggtcttttacagaaagactttgctgacccctgaaatggaagaagactacaggcctagttatttagtgataattgaacccagctttcattgtttgagtagcttctgcatgtcgattgttaagctttacttacctagattacttcaaatcctacaaagtacatattatcgatcccctgagcaaagctaggatattagctgaagccttaaattcaaattcttactttttaaatttaatttaatttaattaaaattttttttttagagacagggtctcgagctctgttgcccaggctggagtcagtggcatgatcatagctcactgcagcctcaaattcctgggctcatgtgatcctcctgccttggcctcccgaagcactgggattacagtgcctggtctcaaattcttacttccataccatggcagaggagcagagcaagacctcttcagaaacatgagctctaaccaaggcagggaaaatatatttagaggtcctgaatactgaaaacattacagtgtaccttccccagccacccctctgtataatccaaaatattaaacattgttgaactcaaaactgagtgaaagcaagtccaacagagttctaattccctccatgataactacatgtttttctaaaatagtatccgactattttatgagaattttttggtgtccctaggtatatacttgcttcatttgttgggtgattaaaccccaaaactgaccaaaatctgttggccttgctaagtctgagctcagggcacagaagaagagtctcacattgtgacagccacctggcgtggcgatagagtcctgttctttccaccaagagagaagccgtccctagagaagtctctcatttaagaaagcagaacatatctactcaaaaagccatggggccacctgaatcaaatgcctgtcagaccttctccctcacctcaggtctgtgtctccctaagcccatgtcatgatcagagatgttccttaaagctgggctccccagcccccaggccatgcaccagtacaggtctgtggcctgttacgaacaggaggtgagtggcaggtaagcaagcattactgatggtaatggcaggtcatctggagtgtctgctgccatcatactggctgcagcaggaatgcgcaagtggggctgtgtgctccatgaagccagcgggaaccagggacaagtgggagctccacctcttccgagttggggctggagctccctgggtgccacttcagctgcccaaatggcagctgcagacccaggcctcttgcagatgggagccccgccctcccaggcatagcaggcagacaagttcctgggcagaaggaggtgggtcctggtgaggccccaccttcaggccagggagggtctgaagtctgtgggcccagctgccagtctggtgaaccagagtggggacttgtgctgccttttttgggctcatccatggccactcattggaccaatcagtacatacttcctcccctctgaggcccataaaagccctgggctcagccagagcagaggaaaggacggagagacactgggatagccagctgcagagagaagataacctctcatcagggaactacagaggacaggacaaccagcctgcagagaggagctaccctctctgctaggagctaaacacttgtcaggacaccctagctacagaggagctgcccactgcaagtcttctttgagctgttctattgctcagtaaagctcctcttcatcttgctcaccctccacttgtccacataccttattcttccatgttgcaggacaagaactcgggacccactgaatggtgaggctaaaagagctgctgtaacacaaacagggctgaaacatgccccttgcttgccacattgtgggtgaagagaaggagagaagagctgcagcccttcagggatcccagacctgggagctccctgagccagagccgtgactccctctttggggttctgtggttcctggcatctgcaagcttctgggtgccactgcattccccagtgccagccagggaagtggcttgcagtgcacctggtccagccacaaccttgcagagagcgctgctggcacctgtagctgcctgccccacagcagccaccagtatgtctgactgagcagtggccggaccccatgctcgctcacacacccctcactgttccacacccgactcacccttggcaggcgtgggacccaggccagcagtgtgaactgagtacagcctgccaggcccagcaggcctgagcaaaacttgggtaaaaacatcactggccacagaggtttctggctaggaaaacaacaccccaaggatcctgtaacattcatcggaacgccacctcccgttagatcagcggtggcatgagattgtcataggagcacaagccctattgtgaactgtgcgtctaagggatctaggttgtgtgttccttataagaatctaagatcgctgagattgatgagatcacttgagcccaggagtttgagaccagccttggtaacacggtgaaaccccatctttaccacaaaaacaaaaattagctggatgtggtggcgtgtgcctgcagtcccagctacagggactgaggtgggaggatcacttgagcccagggaggttgaggctgcagtgagctgagattgcaccactgcactccagcctgggtggcagagtaagaccttatctcaaaaaacaaaaccaaaatggtttattgtaaaaaaaatgagtatggtcaatatttttttctcctcagttctactttaatttcaagcactcaagtgaggatcaagcatctgatgagaatgggagagaaaggcagagagagctgtgtctgttcaggaaaccgcatcctttcacaattagggaaacaacaatttttttttgaggcagggtcttgctctgttgcccagggtgaagggcagtggcacaaatcatagctcactgcagcctcgacctcccgggttcaagcaatccccttacctcagtctctcaagtagctgggactacacacatgcaccatcacgtctggctaatttattttcatttttaattttttagtagaaacagggtctctccagaaaaactacagatggatcagacaattaaatactgaaccctgtggaacaaatagaagagaaagtgaaggcttgtctatccctagacacactctttctggaacatccgtcttcctcacactgtcccctcttgacttccatgataccctaggctgctggtttttctcctacctctctggccagtctttctcagtcttcttggccggctccccctgtttctgagccccaatccctatatgttggagtccttttgggtctcaatttttttttactccttctcttttagggttttcttcctatgagatctttcagtctctagcctttaatgccactgagtgttgccatttctactcccatgttcataattccagccctgatgtctggcctgacacttagagactgtccacggagggatacaggaacaaaggaagtgacaggagtgacaaaggaaaagatgcgtttgtgtgtttctgcacgtttctgtgtctgtttgtctgtgtctctgtaggttctgcatgtccaaaaaagaatacagacgaagaggccaacaacaagggtggacatattgcagcaaacatgaaaaacaaagaattgctaccttatacataaaatgttcataatattagaaaacaaacacattaaggctccaagaataaaacaggcaagaagcagggtcagaaagttctcagaagagaagatacatttagtatacaagcatagaaaacgtccagtcttagaacttatatcaatgcaaatgaaagcaagtagatacatagttatataagaagaacaaaggttgagaggttgtgaatgctgttgttgttgaagcgagtgaaacaggtgctctcccatagcccgcaaactcgtatagtcctgttggaaagcattttgctgcatttgacccagtaattatacttgtggcataaatcctaaagaaatcattccataagctaaaaagcaaacttttaagaagcatctatacagaagtagattaagtaagccttgataaatcactagattttggaatatctcagattttcctgacaatgggaatcacccaaagtacttaccatgtatgcaagttcctctccctgggaaattctgattctgtacctctgggatggtgcccaggaatctatattttaaaaaggcactttaggctattcttatcttcagacacatttggaaaatactgatagaggaaatataatgaaatgccatcatgaggtcattaaagctaatgtgtgcaaagatcgtataattcttttttttttttttttttttttcagacaaagtctcactgttgtcccccaggctggagtgcaatggcacgatctctgctcactgcaacttccaccttccgggttcaagcaattttcctgcctcagccttcccagtagctgggattacaggtgcccgctgccatgccaggctactttttgtattttaagtagagacagggtttcaccatgttggccaggctggtgtcgaactcctgacctcaggtgatccgcccgccttggcctcccaaagtgctgggattacaggcgtgagcaaccatgcctggctgcaaagatcatataattctatggaaaaatacttaatgacattttgagttcctagaatgtcaaatgaaatagcagaatataaaagtctgtgaagtattggtctattcaacaaataaatatttactgagcacctactaagggccagccaggtcgtggggagacagaagagaacaaaacagctgccatttatcctcatggagcttcgagtctaatgggaagataaagagtaaagttaagaaaacacacacacacacacacacacacacacacacaaaattccatacttacctaactgcatggccatgatctctttacaaacacattgtctccttccatgggcggagagctgctgcagaaccaactgcttttggtgggattctagctccattacttagcaagtgcttgcaactctgtagcagcttaggaaagaactgtggttggaaggaaagagtgtggtgcatggatttggtaaaagagtaaaaagagtggctgggcacggtggctcatgcctgtaatcccagcactttgggaggccgaggcgggcagatcacgaggtcagcagtttgagaccagcctaaccaacatggtgaaaccccgtctcttctaaaaatacaaaaattagccaggcatggtggcacacgcctgtagtcccagctacttgggaggctgaggcgggagaattgcttgaacctgggaggtgaaggttgcagtgagcagagattgcaccactgcattccagcctgggcgacagagtgagactccatctagaaaaaataaaaataataaaagaaaaaagtaagaagagtaggagcagaaagaaagtgagttaataaatgaccagggctgtttctgaattctgtatggtggggcagaaaagattttctttaagtagacttctgggtacctgtagacagacgtgctgaaaacccactggcagaacagcagccctggtctggagggaccatgttggtctccagaagctaataccacaggtcagagttcagatcacccaccccaaatctgggatctgggatcagtatgagtctaggactggggcaaaagcccggggtggggatagagggctgtgtgaattgacctgccattcagaaacagcctcaagtttaggcttggagttatctccaaatgagattatgaatactgtcacagagagccacccgtaagatcgaaaaaaaaaaaaattaaccaggacttttacacttgtgtgttatgactgagctgtattgactctgatgcagtctgaatattttaaaaataaatcatacgcttatctgggaaccaaaaaaatatgttgcattatagttggttgaagtaaatatttaatatcctggatatgatagtttttataattctgggttggcatttcttccttgtatcaaaaactatactaaggccagttgcagtggcttgtgcctgtaatcccagcactttgggagcctgaggtgggcggatcacctaaggtcaggagttcaagacaagcctggccaacatggtgaaaccccgactccactaaaagtacaaaattagccaggcatggtcgcgtatacctgtaatcccagctacacgggaggctgaagcaggagaatcgcttgaacctgggaggcggaggttgcagtgagcggagatcatgtcattgcactccagcctgggcaaaaagagcgaaactccgtctcaaaaaacaaacaagtaactatattagaatcctcaaacgctggaagtggtttaagcctgccctgactctgagaggctattccagggtaagaatgctgcccagtactctcaaaccctgtagaaaaggggctggtgcttatttccttagaggcatttctgtgtagtttatctttggtgctaatgcggtccttttcaacttaccgtgttaaacaggacattagggttctgttaagaagagatgcactttgggaggccgaggcgggcggatcacggggtcaggagattgagaccatggtgaaaccccgtctctactaaaaaaaaatacaaaaaaattggtcgggcatggtggcgggtgcctgtagtcccagctactccggaggctgagacaggagaatggcgtgaacccaggaggcggagcttgcagtgagccgatatcacgccactgcactccagcctgggcaacagagcaaaaaaaaaaaaaaaaaaaaaaaaaaagatgtcgctgagtgagggagaacctctcctgggatatgtcctaccaggaagcatatctgcaggatcagattacacagattacaggaggtaacagagctggggacttagaaacagcagctgtctagtttcctatttatttactcattctgagcactgtccattggaatttttttaggaaggcaggtttggtgtgggctaggtagttgagatcctgagacctgctggtcttgatctgtagggagctgactggatgaccttggccccaggcctgccatagatgtaacagggaagatgcacttggccatctccaagggccactgcagcccagaacattctacgttaataagactcaagagtgtttgcccaatggcaaaaacaaaagtcacaccttccaactcagaccatccaaacggtttatgaacttccaagttttatttgttgaatcccacaggtctatcatcattgtaaactcttattccccccagtaatatatctgtaataatcctgaagcatgaatatcttgaaaatagctgcagatgcctatattttcccagcagagccgataaaagagacttttgtttacatattcatcattcagagtgctttgagaaattaggaagtaaatcgagttgcaattctgcaagtgacttggcccttaggactgtcttacagtgtgtggtgtgtaccttgtgcctattcaggaccattcctatcaaaatgaatttgtaatacaaacatgtcttcagccaatgggaccacagaatctcaccttgtcataagagatgcaatcagaagtattgtgcaaacacctttccctgacagaataagttcctggcaacccagtagccccctgcataatcaaacagtaagccagatcctaaatgttctatataaatgtagaatatggaaactgtagtcaaacaaaaatagcaatagtggggtagaaaccaggactctgtacttctgtatttcagtccttgtgtccttcagtccttctcaggccacgtttagtttgttttaacaacctcagcctagaactgcccttaattctggcaacaagggccctcctctggccccatgctttcaaggatctgctctcctgcaggtgtggctcctttcttagggggaaatgccgggctaaggaatgtatccctcaaggcctgggcctccctattttagaacattctctggatacccaggattccccgctcaaatgttctgggcctatttctaggacctgcccaggttctttgcttggtccatcctcctgagggcagactatactgaagccttaggctaaagaaggggcagcttttttgtggggagacggccagcagaacttggacctgtgggccgagatgtgcacccaggtgcatgtgaggactttctcagtgcaagatggagctggagggagtgggatgggaaaggaggtggtatcatgtgctggcagctggctctccccatgccaacgtgttccgggaaaaaattccaaggagcctgagaactcttaacttggatctagtcttctaggtcataaatgaaggtgtgcatatatatcaaggtagaaggatatgttatctttaaaagttttgttagtttcagccaggcatggtggctcacgcctgtaattccagcacttcgggaggccaaggtgggcagattacctgaggtcaggagttcgagaccagcctggccaaaatggtaaaaccccatctctactaaaaaaaaatacaaaataattagctgggtgtggtgacgggcacctgtaattccagctacttgggaggctgaggcaggagaatctcttgagcccgggaggcagaggttgcagtgagctgagatcacgtcactgcactccagcctgggtgatagagcaagactccatttcaaaaaaaaaaaaaaaggtttgttagtttgattggtaatgtttaaatatttagacatggagtaggtgggtctcccacttgtgatcttgttctgagtgaaaatgttaggggctgagctgccttaagcaaatctcttcacctctgaggcttggagctcctctgtaccaggaagccttgggctccttgagggctactggccggtccagctctttctttctttgaatgttggctgatgaggctgaaactgatgaagaaaaatgtaggcaacttctttccatggctgctttaggtgggattcttttcagtgcaagggacaacaatctaactcaaatcaccttaagcaaaagagagattctttctgttcacttgcttcagacatgttcatatttagttactcaaacaccatgttgtccataatttattcctatttcttcttctgttttcgttttttgagatggagtcttgctctgtcacccaggctggagtgcagtggcaggatctcggctcagagcaacctctgcctccagggttcaagcaattctcctgcctcagcctcctcctgagtagctgggactacaggcatgcaccaccaagcccagctaatttttgtatcttcagtagagatagggtttcaccatgttggctaggctggtcttgaactcctaacctcaagggatccacccacctcagcctcccaaagtgctgtgattacaggcgtgagccaccatgcccggcccctatttcttgactcagctttttttctctattggcttcattttggggcaagccaagatggccacaagcacctccaagcttgaatttggcaacttcagcaaaagagaacattcctttcctaataggttcagcaaaaatcctaactaagcctctcattggccctggctgggttacatgctcatcctctaaacaaatcactgtgactcaactgccaggaagctgggggagtggaagacggcggactcgcctgaaccacagggcagtgtggggcaaagggtatttccaacaggaaaagaggggttctgatgctggaagaaggatgctatgtaggcaaaatcaacagatgtttcaccagcaatgcttaccacatgaactatgaggacaaaggaaacagaaacatacaaatatttatgaaagacagcgatgaaatggtgcggtggaaaattgtgctagagaagccaatcctgccccctcaacgcagccacactgagcgagctgtgggtcaggggtacccaccctaccctctccttggctccaaagcagatgttcactacagtcaacttagacattgtgactcagagactgcaagttctgtcagacacttggactgaggatctacatggagataagcagagaaaggtggtctgtgagagaataaagcggaaatgcaaagaacaccagagaccaggcagccccagatagaccaagagctatgactccttccctccagccagtggctccagtgccttgcaaggctcagctgtatttcctgcccttggtagagactcctgggtccctccaacatgttttcgcgcgcgtgtgtgtgtgtgtgtgtgtgtgtgtgtgttacagctggatttaacagtttgctgttccacaaaccacaaataaaacaaaacacaataaaaacataaaggtggggaaatgctgttttttcttctaacatgtaagaattgagtcaggtgtttctcaagactgttgtgatttttatcttagtttttcacaaacatccagagaagggatagggaagcgtgcacgtggaacgacaaggcggctgagttcaaggtctggagcaagaagctctgcatccctgcagctctgatggggacggagaccctctgggcagagatatgcagggaaatgctcattactctgtaccccctaccccaacaccgcttttgccaagaggtggactgtgctagcaccaatgtggagagttttggacatccacgccatatctgtagcagctgcggctatctcaatgcataagctacattctcaaagaatttcacgtcaaaccagtgtttataaacggagcccgattttcagtgcttggagagaacctacacgcttccgttaaaatctctcttctagaaaagtgaaacacaacctgttaatcagcatttatataaggcaatattttaaaaatcagaaaaaagctttttttaaaaaaggcaaagttgacaagacaaataagctggatgaatcaaatttctgctttgttctgctttcactaattgctgacagagccgagttgcggcctgattataaagctgtgcttcagccaccttagcaaatctgttgctggaagacaaggagcgagcacttactttttgagagtaaactgtattttattttttattatactttaagttttagggtacatgtgcacaacgtgcaggttagttacatatgtatacgtgtgccattttaaaagcaccgggggactggtctatttaaaagaacaatggggtgagtggcgctctaatgacggactccagcttgggggctttgactatcctagttcttcttgggccccttttggctgagcgtgaagcaaataaacaaacaccccgatggagaggtccttaaccacggtgtgcagcagcatcacctggggagctgtagcccagtacacacgcccagccccacccaccagccttactgagaggggaagggatcctgcctgtgtgagctggaaaagctctccaggtgattccgcttcaagcttccggttaagcacgaaggctaatgagccttatttaaaagctcaggtttttactcagcaaaatctgttgcttttaaaatggaccgcctttagaaaaaccagcaatgttgcatgccaggatgggactctctccccggaaatgaaataagcaacccctgagaaacggcgctgggacaatagggcagcagtttctcctcacgtcctaggagggaaagtcgactgcagggagttatatgacttaatatgcagctaaccagccttttaattaacttgacatgccagataacaaagctattactaagtgagagtttcttaattgaaagggggaagagagatttgttttatattttcaaaataatctataatgagcgttactaatttgacaatcagaatttgtgtgtgtgtgaaaaatagctattttgagctatgaaaagggaggatgagcagacctgcacacggcagcttagcttgctgtggttttgccttagctggtagacggtgcctggtagtgcatgactgaaagatggtgtggttgattctattagtgtgcaattgttcgcaggcattttacctagaaatcacttgtgccatcgtggccatagtatttttccagcctcatctcttactgaactgtacctctagctctgagtccagtcacaatgaactaatttgtagtctctcagtcatccatgctttgcacatgcagtttcctctctatggaatatgaaatacctccccttccctcctcttccttcccttcagcttccagactcctgccagcaagcttataagtcacctttcaaatctcagttcaaaagcctcctctgagaccatctctccacttgcaagactcgggggctccatctatctcctgggatccctcgaccaggcactctagactgtcattatagcaactcattgagtgtattacgatggtgtgcttttgtgcctgtctccccaccattcatatagtcaacacgcacttggtagatgtcatcatttgatcactgcagcaatcctacagggtaccttttactgtgactcccatttcccagtggaagaaactgaggctcaaacatagtagcctgcccagctctcactacaagtagatggtttacgtgtgatacaatccaggttcatcttgcttctgagtttgtgctcttaactgccatgtgagcaaacttcaatcagaaagtgttttttcttttttcttttctttttttttttttttttttgtgacagagttgctctgttgcccaggctggagtgcaatggcacaatctctgctcactgcacctccacctcccaggttcaaacgattctcctgcctcagcctcccgagtagctgggactacaggcgcccaccaccacacccagctaatttttgtatttttagtagaggtggggtttcaccatgttggccaggctggtctcgaactcttgacctcaaatgatccaccttggcctcccaaagtgctggaattacaggcgtgagccaccgcaccctgcctgagagagactgtcttttcgaatttgtatcttcaatgcccagcctacaggagatgctcagtggataatgatggataattatttagcagttatccattgccaaaagaatggataacatcactgctaccggctttggcagacctcactccaggtaaatcattccctgggggcattaattacctgctggtgttccctggttaaaacacctgtgacaccagcctacacatacgcacagggctctgaggtgattttttttttaatgacaataaagacataaaaagatataaggtaaacctacgtgggctgcttatagcactgtcagttatgtgtgtgttttcatttacttcaaaaactgaggatattaaaataaatatgactttattccatttagttgagattgtcatttttttttaatttggaagagaatttaagaaatgatgactttattaacaacattggcgtaggacagtagcagactgggttaaaatactgtatcaatgttgaatttactaaagttcatcactgtagtacagttttggaagagaatatctccattctcagaaaatgcacactgaagaatttaggggtaaagggctataatgcacacaactgactcggatgtctcagaaaataagtgtgtgtgcatgtgtgtggtttgtatgtacgtctgtgtatgaggaagtgaaagggactaatgttaacaatagatgaatctgtgtgaaaaataaatgcatattctggctgggcacagtagctcacacctgtaatcccagcactttgggaggttgaggcaggcggatcacttgaggtcaggcgtttgggaccagcctggccaacacagtgaaaccctgtctctactaaaaaaaaaaaaaaaaggctgggtgtggtgacatgcgcctgtagtcccagctacttgggaggctgaggcaggagaatcacttgaacccaggaagtggaggttgcagtgagccgaggtcgctccactgcactccagcctgggcaacagagaaagactccacctcaaaaacaaaacgaacaaagaatggatgcgtattcttcatattattcttatttttgcaaattttctgcaagtttgaaattatgtccaaacgaccttggaagaaatgaacatccctgagaggaaggtgtaatgagagtgtttctttgaaatacagtgagcaagagctggcagggccggtcagtgtctgacagtggcatgaggtttctttcaggctgacttgcaatggctggttttctttacctattgatgtgtcttgaatatgtttacagttcagctggcccagttctctgagaggcaattgggtttccttgcagatgtgccgcgggaaggacagtggtgcctgtgcttggagaagcccctggccacgtgctaggacagagggacatatggtggcacgactccagccacagatgcaactccctcaggaacagtggggcctgcagttggaaggggccccctctggctcacagtgctgtgtggacagtagcatctgtgtgactgcaaactcgcccactgtgagtgggaacagtcgaggctatctgtggccttgcatctgctggtcccattcaccagggcaacactgtgcatggccaattctagacctcccggacgcagtgcatgcaactcagcgttagaatgtcaatttcgaagtactagaatgtcattttgctgttacagtcaccccacaagcattttctgagcatcttctacttgggattgcatcctttttgctagggactgtgtcatgtgcgtacacacagcatcttatttttagctttcaggctgacttgattgaacatggtgcagttaatgtgccccccattttccaaaagtagaaaactgtgacacagaggttaagtggtttctgaggtaacatagaaaaaatatgtagcagagatttcctaaacaaacttgcagcctggcaggaggggtaagaagatccacgaggaacattggatcaggttggaggaaagaggtgccaagagagacccaagatcttggctgggaagtgaaaaggagtgtggccacttttgattctggggtaggaggctttattggggaggtggcatttgcgtggagactaacaggatgataagaattttgaaaggaaaatcataaagagctttccaatggagtcgagaaaacatggtaaaaaaacaaaataggagttgagatcataacaactgtcatttattgagtttttctatatgctaggaactgtgagaggcgctttagataaatcaactcattgaaacaggagttttcttaagtgagccctattagcatcctcattttagggtaaatggaggcatccatggaaggttacatgcatctagtgtggtaacaaagcccacaagcttagaaagtgcttcatgataatagtgaaatgatggtaataataggaaaaaggagggggaggaggagggagaggggaagaggaagaggaagaggagtggggaggaggagaggaaaaggagaaggagaggaggggagggggaggaggaagaagcagcaggaggaagagtggaaggagaaggggaagaagaaggaggggcaaggggggaggaggatgagaagaagggagaggagaaggagggggaggagaagggggaagggggagaaaacaagagggaggagggggaggaggagaaggagggaggtaggaggaggagtgggggacaaggagggaaaggagaaggggaagagggagaggatgaggagggggaggtggaggaatgaggagggagaggaagagagaggagaggaaggagaagggggaagggagagtagagaaaggaagaggagggaggagagggaagaggagggaggagagggaagaggaggaaacgagaagaggggagaagaggagggaggagttggggaggaggaaggggagaagggagaggagagggaggaggaggaatgaaaataggcagggggaggaggagaagagggaggatgggagaagaggtaggagggggaggagagggtggagtggggttaggggttagtcctggaggcatcagaggcttctctagggagcgtggtttctatcctactctaccttagccttgaccaagcaggcagatagcattagtattcactccttgcttgggagcacttgaaaagtttataaaaaggcgtaggctgtttggataaaagatgctctggagacaagacagtgcatcttcctcagtcacttcctcactcctttctcggctctgattctggtgtttgatgtcttcccacaactcggcaaagaaagaagaaaatccctctactcactgtgcagtttgtaggttatttaaaggaaatgcattcaggtggttccttacccggcagggtgcagggatggagtgggatacaaccatacaaccaacccctcagagggcaagcgcagctcattcacagtggccaggatccctagggcagcctcgggcgtctgtcccgcagcagaggacactctcatgaggcgctggaaactcagctcagggcgtgccaggtcccacgggcgccttccagcctgggacacctgtgccaaacctgaacagggaaggtgcagaaaagcgtgtgtgtgcgcatgcacgtgtgtgtgctaaaatataaatgaacgattaagggtttcctctgctggatattctctgcagtggggagaagaggtgggagaaagtagctgtttttgccgcttggggaatgtttgcccaactggtaaaggtagaattgttcttttccaaaggaaagttgtgtgggagttgcttccttaccgaaaacaaggaaaagcattagtgaaaagatgtaagatcaacaggcaatcaaaaatgcacactgccagtgttaagggcacaggtgaattttccttctaggattctcaatacaaacctattttgaaataaaatgcctctaggtcttccctgcctaaacccacgtggggagcactaatagctgcgtacaaacttcattaaactggccacagctgaaaggagctggtgccaacccactgctttttgctgaccgaagtatccggctgggtttttgccctcattctgaagtgactgctgcccatcccccacaccttgagcattgttttactagacatcttctagtgtagggtaactggaagaaaagtaatggaataccaagtgccattcatcatatccctgcctcttctattttgtggtgcagggatgctgaggggaaaatgagtctcctgtaagtgcttggagatcctcccccactccacctcctgcatttccataagcatttggcatcagagtcttctggtaaaccccccagcttctacaattggacaattggctttgtatcacggcaggaattcgtgcctctgaagtttctagggaagctctacagaagcaataaagtggtagagttgtttgaataaaattagcttctatgcttgtaggaagcatacccaattccagttagctgtatgaaatgcaaccattttggaggtttgtgaaaatatgcaaggctcccggcttcaggagaaaaacagatttacattcctccctgtctcagcagggagtcttcaatcaaaggcaaccaacaaatcaaacatgattatctgtcagcacattggccctggtttgtaattatacatttatttgtgtgtgatcaatgctagtctcctcactggattctaaactccctgagagcttttctgtcttaattaccctgaactccagtgcccacacagtacctggcacatagctcatgctgtaaatatctgtggaaagaaggaagaaatggagaaaaggaagggaggaaggaacagaagggagaaaggaaaacggaaaaaaagaaatgttccaggtggaaggatttttttttttttttacaatcatcctgcccaacagtatataggtttgcctgtgatctttttctcatacataagatggagataatagtccttgtctcaatagttattttacgttattttctaactcaaatagttaaaagtcatttgtaggcccctgctctgggcccatgctttgtaggatctcactgtcgctgtcctcaggctgtgccccttcctagagtatgaagtcccggtgggactttaagcctatgctccccttccccttcctccgcatctgtggggacttctccccgacagttcacgcaggtctccaccacaagtgtgcatgccctaggcccaaggggtgtccaaggagtgactatttgtaggggatgagccatggatggaactgtggtgtctgcacacatgtgcctaagaccctctcccattgtgggatggagcctgcagttcagtagggggaatgaagggaggtgtgaatcatggctcttgacccaggcccgcctctctctgtgtggccagggttcagggcagaacctcaggaggctggaagttgtagcttctaacctggcctttcaggtcatgatgaaggtctatttgtcagggtaagaggttcaaacctcctgcaatagtcctattcagcagctgatagcttggtttataacttttgaatatttagatgtattccacgtgggcaaataggaacacacacacatatatatgtatatttgtgcatttatatgtgtgggcatgtgtgtgcacgtgtgtgtacatatataattctatagttcacctgttagtgtaccttgatgatgaaaagtgagggaggaccctgactttggacagcatggatctgcctgccacttaccagctaaactgtttccttagggcaaaaatagagacaacaatagtacctatttagttggattattgacattattaaaagagagcaactaacatactcctagaatataagtgctccatgcatattataaactaacaattgtttcctgctcctttcacttcatgcatgaagacatattcactcactcataaatacttgcattatatctatctatctatctatctatctatctatctatctatctatcatctatcaacaaagtcttgttctgttgcccaggctagagtgcagtggtgtgatcctagctcactgtagcctcgaactcctgtgctcaagcaattctcccacttcagcctcctgagtagctgggactacagatgtgcaccaccatgcctggctaatttttgcatttatttgtagagatgagctctcactatgtcgcccaggctggtctcgaactcctgggctcaagtgatccttctgcctcggcctcccaaagtgctgggattaggagtgtgagccaccatactcggccattatgtatatttcttattcaatctgagaactaactataatattattcatttactattttagttcaagttgatttccttttaaaacatacacaccaagtttatgtgtattgataccagtggtttcccaggtgtttttttgttgttgttttgttttttcagattctcattctgttgctggagtgcagtggcgctatcttggctcactgcaacctctgcctcccgggttcaagcgattctcctgcctcagcctcccgagtagctgggactacagacacgtgccaccacgcccagctaatttttgtatctgtagtagagatggggtttcaccatgttggccaggatggtctcgatctcttgacctcatgatccacccgccttggcctcccaaagtgctgggattacagacgtgagccaccatgcctggccttatataggtatttcacaaaatgatttcctctattaggaccatattcaaaaagcccttcccctactccacaattacagaagcagtcacatacattccatttgattcttctctatgatttcatttttgaaacttaattccttaacccacctggaatttattgcggtgttgttgtgaggttaagaaaaaaaaaaatcaatctaatataatgtttctaaaaagccagttgtctcggcatcatttttggaataatctttcccctcatcattcatttacatttctacctttgtcacatagttaatactttttttcaatttgggtttctttctaaacctgtaagtcaattttaatgatctagttaacttttgatgccagtatataccgttttaattcttgcaggtgcataacagttaatacagcagagcgcaagggctgcttagttttcttgtttttcccttttattttgggtgggttggggaagggaacaaggtcttgctctgttgcccaggctggagtgcagcagcgtgatcacagctcaccacagcctcaacctcttgggctcaagccatcttcccacctcagcctcctgagtagctgtgattacaggggtgcgccaccatgaccagctaattttttttttttttttttgtaaagacagtggtcttgctttgttgcctaggctggtctcgaactcctgggctcaaacccacctcagcctcccagagtgctagaattacaaacatgagccactgtgcctggccatttttcttctttttcaaagttgatcaattatgtgagcatcaccactagaatctgcaaatgtctcctgtatcggcaacgagggaggtaccataagcacccttcttttacagatgaggaaactgagcacagaaagaagagacacttgctcaaggtcacaaaaacaaggcaggtccaggaacagtgaaacacaggcagtctagctgcagggaccacgatcataacctctgcaaagtggggcagatccaacctgagaatcaatctccttcaagtcggagcattttctcctcatatctattattactgacttcttagtatttgttttatttatttggttgtttaatgatttcatatgtttccctgtgtttcgttatatactttctatttataatgcttcttaaagttttctggttacagactattttctttctttttttctgagatgtggaacttaccatggttcatattttaaactctttggctaggtttactaataattgtgcttacccgaaagcattctttaactgctatttctttggttttcaaggtcagtgactctttatatggctgcatacacattttagtacaatgataactggataattttaataaagttgtataagatatagtttacgaacataaaaatgattctattattagctaaaatttcagcagcactgttgacataatttttattgttttaattaaattgcatggaaaagaaataattttatcataagaataaagaggatgatagttcaaagttatttgtgagaatatcgtggctgtattgcattagcatcttgacttttaaggtgatgtttaatagagacacaacaattctttaggtcgtaaaggcaattcttgctgttttaaaaaaatgttatgacaacaggtgtgatcacataaagtattagtaaagatgaaacaattttaaatattttccactctatattctactgctttataagaaggctgacaagaaaaccctcatttcactagatcatatctacatctcactggcaggaaagaagggcccatatgagttacttacctaagtaggaactattattcctgttttacagatgagaaaaccaaagctcagaggctaagtgactagttgaatgtcagcagaccaattgaagaaaactcaaaatgtcaccactcaccaaattcacctgtctatccagccagtgcacacatccttggcagatgtctcctaattaagtggagtgtgtgtgtgtttgtgtgtgtgtgtgtgtgcgcgcgcgcgcgcgtgcgcgcgcagtgaggtgggccaccccgcctgcaggcagctctaagtcatagttccgttaattatttattttatatgatgattttgagtccttttgtagtcctggctgtctttttatgagcacatttctatttgagaaagtcagcaggaatctggattctggaatcactgaattccaatgctagctccaattcttcctagaaacgtgatcttagaaacgttaatttatataacagaaatgataatacatatcttacaggtatggtgtgagagttaaatgagaagttgtccatgtatttagcattgtgcctgactggtatcatgtgctaatgcatactgctcattttattttatttccatggtatggacgtccttttaagaatattcgcccactgtagctgggcgcggtggctcacgcctgtaatcccagcactttgggaggccgaggcaggcggatcacgaggtcaggagatggagaccatcctggctaacacagtgaaaccccatctctactaaaaaaaaaaaattacaaaaacttagctgggcatggtggcgggcacctgtagtcccagctactcgggaggctgaggcaggagaatggcgtgaacccgggaggcggagcttgcagtgagacgagatcgcgccactgcactccagcctgggcgacagagggagactgtctcaaaaaaaaaaaaaaaaaaaaggatattcgcccagtggaacaactttggctgctggtccctcctctgtctcccccaagcagggttatatagttcgttgagacattcccttcaccaaaaggcattcctcagctcagggaaaggaaagtggagaggaatggtgagtgagaccgtctttaaatatcctgaactactgcccccttccttattgtctactatctacatttggggagtgattctcttagcaacctctcaggtttgatatcagcaatactgactcatgatactaccccaaagccaaagcatgaaacatggaaggtgttcactagggacaataccagatttccttaaatcacaaagcaacagagcacatcacactggatgtctcactctggcttcctgcccggctccatatcaacgggcaattgacgttggggggagccatttcctactctggccttcagcttgcggtcagctgagtgtgttggaccacacactctctagcatcctgcgattctaaccttctatggatttcatcagttttatagatatgagttcagcctacgactttgggaaacaaaggattcaactgtaaaaaacatttgaattccactgatctattttatctctgctcaggaagaaaaaatggcaccttcttcctgaagtttgtgtttccggtctccttgatttctgagagattttaaaattactttctatttttcttactctgttctgatattgcaaaatggttattaccaattattaactaagtgatgtttaattttagaagtcaagctacttgtaagggcccatataaatgtgtgctaggattagctttagatttgttttctgcttctatttacagcaaggacaggactggggagtggttttattttattaagctttttagcatgatttaatttttaaaactcaggacgtattactttaaaaattaatcgaataaagatgtatgttcataacttgaaccacacagaaaagtaaaatacaaataaaattgtgatctcattacttaaagaataaccattgttggccatgtgcggtggctcacgcctgtaatctcagcactttgggaggccaaggcgggcgcatcacttgaggtcaggagttcaagaccagcctggccaacgtggtgcaacctcatctctactaaaatacaaaaaaaattagctgggcatggtggcgtgtgcctgcaatcccagctacttgggaggctgagccaggagaattgcttaaacccgggaggccgaggttgcagtgagcagagattgcgccactgcactccagcctgggcgacagagcaagactccatcacaaggaaaagaaaacaagcattgttaaaattttgatgcaattccttgtagcctactcattcactgtttctaatgcttactaagtgtttagtaacacatacatacacactgcacacacacacattgtctccttcttcactcaacataaggatagcatttcctatattattaaaatatttttaaaaatgtgtgtgtgttacatgtgttatatgtcacacacacttttaaccacacaaagacacaggagaacatcaaaaatcaagatgctttcacgtcccctcacacatgtgatccttataatcctgtgtgagaagcaggactggaaatatttccaacttccagctgaaaatgcatagctcagagacaggaaggaacttaacgttggttaagatcacaggctcggggtaccacataccagctgtgtgaccctgggcacaataatggatctaagatttgtggggcgcgaagcctgtatcattttaggggttctccttaaagaaaataataaaacatttacctgtgaaaattttagtgatttcatgtgatcttgtaagtatattgctaggacctcttccagggccttggaagggtctgtgttaagtgaggagccctgtagcttcatttcatctgcttggaggcaaatctgcctttatttgggtaagtgacttattttcatctgtaaagtggggataataaaagtgcttgcctctgagtagttagaaagattaaacaagatactgtattgtaaagcattttgtaaacttcctggcacattggcacataataagtgcttaataagggtcacctgtgattactaattttattcaaaatcatgtcattgtggctggtgtcatttgagctgcttcccagagactgagcgattcctgtacatacctaaagttacaccttcaagatgctgcagcttggctcactcactcatttaataagcatttaggagttcctgctagatgctatgcactgtgctaggctccagtctcaattcattctcacaccacattcactggaagcacaactcaggtatcccctcctctgggaagcccttctaggaccctaagccgactcactactatctgggcacttatctctctgtgtgactgggtttggacatcactagtattcaaggaaaagacattatcctgcccctctgccacctttgttcatttcagttcagtataatcgatacttctctctgtgcctataatacagtatggaggtgctcaataatcttaaatgagttgactgagcatgtgtttgttttcacaggaagatttccgtttcttttgcaagctatttaatttgcaaaagtaagcaagatgtgcacaaaatagttttgagacatctggaaacaaaacaaggttgcctcatcattaatcttgtttttgtgtgataactttactttttctcattttatgacaactgaaattctctattatactgccagacctcattctgcaagcttctctcctgtgctaataaaaaatattatggccacatcgagaagtccttagggaatgtgttctgcatcaggaaaagtaattaagctctggggtcctaaaggagcctgggaaagtctatccagaaactatggggttaggatgtattatctattgaaaaacagaaccggactttgcaagttttacaatatcttggcttattaaagccactaactgagaattaaaatttctggattgttacttttacaacagcagtcaagtgtcggaaaatatcctgaccagtcagtaaggtatacaaatagagaaggcaaggagtagctgtgagtaaagcgccaactacatttgctgagtacctgggaatttacgagttagcttttgctatcattatccgtctcgctaaagcaaccctatgaggtaggtgggaagctggatgccgtcctcttttgacagccaacactgaagaacagctggggctggaaactagatctgtcagacatagtaactgcttctatcactctcaccaccctcccatgctcttgagagtgccttcgcttttgtgggtgtcttcagaaaagcatgcggatctctgtataggttttactcaagtgttcctctctgtggagggtgacctgggctacatgaacatgggcacctcaggatcggcagctttccatgaattcctatggtaaggggttcagcttatccttcatgtgggtgaagatgtatgatttcattgaacattggcagttacagccaagtacaagtcctgccttcaggatccagcagggaagaatgacattaaacatgtcaccttggagaaatgttgcattcaccttccgggtaatgacccagccacccagggactcctctgaaatatccaatcctctaagtttaaacacgtttcagaattaatccatctgaattcttatcgctgtagatgcaaggagaaggagttatggcaggtctgaaactattagcggccaagctccctagcagaagcaacctctccctacaccccattatccgtgcacagctccttatcagcggaggaacaactttactgtcaccatattttctacttggaaaaaaaaaagaaacctcagcaggcccaatccgaaggctatgaaatttcaaagaaacagagctaagaggcgagaaactagccctttgtgttaaaaagatggaaatgctccaagcgcctttccagtctgctttctgtttacaggccttgcgtgagcgcgggaggctgggcctcatctctggctctccccagccaggaccccttactcaaaaccctccatctcggcaagaaccctcattcccaagttagttggattccaagtccataaaccgggtcaaaagaatacagtaatttcctactggagctctaagtggtggttttcacggaggactcggcaccatcctcccacctgcctcctcccatcgaacattcctttttaagaaaaacacacaccaggctccgggaagctgacgtaaacatcctgaggaaataaccactgtaagtggcttctaaacccatttccccaaggaaataatcagcacctctttcccaagacagctccaggtaagcaagcggtgaagggagctgcaccaccgcgttctcaaaagtaaaggcgcttgcggaactgtctactgatttgtaagcgcgcgcccatccactgtcgcatttaatcttccgaacgacccacgaggtggtaaaggcggggattattttcttcattttacgggtgagaaaccgaggcccacagcgctcgttcctgtagccggggtcaggcagggcacacctaggggagcctctgccttcgagccccgggaccgccccgcggcaccacgagatctccccagtcagcccgtgtgcggctgcggccgcatggcctcattgttttgggaagacgtccctctgtgaggatcttgggcgactctatgaaccgcgggcccagccgctctgcggaacgatccgcagcgggacgcaaagggcgcggcgagcccggcggctcccggaacaaaggacagcagagcgcgcggggcccgaaggggcgtccgccctagtgggcggcggagggggatgcgcgcggagaggaccagcgcgcaccgccccggcccgcccctcaaatcctccttccttctctctcgcactcggagacggtccctgggagatccgggagggggcgcagctcgccgtcctcgccggcaagtgccgtcgcaacctccctctgccgccacccccaccccgagaagcgcacaaagagcggccgggcagggagcgctcacctcccgtcggggcggggccgcgggcggggccggcgcgcgctccgcagcgcccgccttaaagggcccgcccgctcctcgcgcgcactgcgcatgctcggccgcggggcacggaggggagggatgggaacagcgggcgcgcacgcccgcgccgcccgctggcgctgtggcctgcgtccccgcggtggcggcgcggcgctcgtgcgcgtgtcagaacccgcagggtctcggcccgggcgccgggcgtgtgctggacactggtgccatgcattccagaggtcgccagcggccgggcgggccgagctcgcgcggcagccagcttttagctttcccatcctcagtttcagggccagttgggcgaagtgctgcccaaggagacagaaatgcaggcgcgggcgcgcgcgcgcgcggttgccagtgtgggcgggcgtgtgcttttgtgtctcgtgcgctcccgcgcaggtggacaacccgcgccgggagtcactctgcccgtgcgccccaagacctggagtcccgttttccgtgtcggagggctcgggtcgcccttttgggcggactacagactcttctcacagaggaagctttggctccacggatggtttatttggagccactaacgggacttcctgaggaccgctcttttagagcccggctccaggcatcagagttgggcgcgttttcttttctcagtcaggcgagggaggagacttagggacaatgattgtcctcggctgataggtacatccaagtgtcccgagcctgccagtcccgcattagacaacaaagagaggcgttagcggcggcgggggaggggcgcggccgggaggaggacggggcgggctgcggcgagcgcgggggtggggggtggcgctctctctccgctcgctcaacccgcggcctcctcccgcccccggcctggcgcgcgccaatcgcctcccccagcgatagtgtcagtagcattgtggtgtcagctcccgcctgtgacgttgcgcctccctcgtccccctccggagtcgtctggctgcagaggctc

SEQ ID NO: 3 - DNA, 836 bp, Human
gtaggtcgaggagggatggggaggtgggtgggggtggtgtagggtctcaggccactgcctcgaggggaaggcgtgttcagtatcgggatccgcggcgtggggtgccttggggagagaggaagagccgcgcgatgggccggcgccccagacaaagaaagtgcaggcaggctgtctcccggagccgcgccgctgccctggcgggatgcactttcttctgctaaaatcactgccttctcccctaacgccccccaaccagcccacctccagaaagacaatttaaatgtaagatgcttgggggagggggcctttgatcagtcctttgggaggaggaaggaggaggagtgagcataggatgggaggaggattctggatttctgcaaagcggaatggagcccagaggaggaacaatgggtcccgggactcacaccccaccccctacccccagtcgaccagcgctgaggcatcgcgacttcagctgccttccccgagccccttccccgtgtcttcagagctgacggcgcgcccagctggatcccagcggcatctccccagatgacttttctgggattctcgggtttggttcgggacgactgcagtcactgggggagggccaggcagccaatgggctgttcctcgagcgcctcgcgggtgggatccgctgcccagcccgtggcgcggcccgaggtcagtgagggagacgccccctttccgcccatctcttgtcctgccgtctcgctgtcctggacgcgggctgtccccggtccccgcggttaccccaggataatgggcgtgtctgtctctctctcccactccctcctccgcaccctggttcgtag

SEQ ID NO: 4 - DNA, 3416 bp, Mouse
tgttcgctttgcgctcggcattgtggccagccagccgggcactcggggggcacgcgcggccgccgctcgagctctgcccccaccccaaccgccagcagatctggggtggggacccaggcgggggctcttgcagccactgcccggtgcggattgcacgcagagacccactcctccgagcgccgaaaaacgagccacggagccctccgcagccgaccggcctccccgcccctgactgccggcttcccggctgcctttgtggctgcaccttctagctgccgagcagagagccggctggggcgcggcgcgcacggcggagcgatgcccagctcgctgtttgcagacctggagcgcaacggcagcggcggcggcgggggaggcggcggcgggggaggcggcggtggcagcggcgggggagagactctggatgaccaaagagccctgcagcttgcgctcgatcagctctccctgttgggactggacagtgatgagggcgcctctttgtacgacagcgaaccgcgcaagaagagcgtgaacatgaccgagtgcgtgccggtacccagttccgaacacgtcgcggagatcgtagggaggcaaggttgtaaaatcaaagctttgagggcgaagaccaacacttacatcaagaccccagttcgcggggaggagcctgtctttgttgtgacgggcaggaaggaggatgtggctatggctcggagggagatcatctctgccgcagagcacttctccatgatccgagcctctcgtaacaagaacacggctctcaacggagctgtgcccggaccgcccaacctgccgggacagaccactatccaagtgagggtgccataccgcgtggtagggctcgtggtgggtccaaagggcgccacgatcaagcgcattcaacagcagacacatacatatattgtgacacccagccgagacaaggagccagttttcgaggtgactggcatgccagagaacgtggatcgcgctagagaggagatcgaagctcacatcgcgctgcgcaccggtggcatcatcgagctgacagacgagaacgacttccatgccaatggcacagacgtgggctttgatctgcatcacgggtccggcgggtccgggccgggcagcctctggagcaagcccaccccaagcatcactcctacacctggccgcaagcccttctccagctatcgcaacgacagctccagctcgcttggcagcgcatccacagactcttacttcggtggtgggaccagcggcagcgcagctgctacttcacgcctggcggactatagccctcccagccctgcactcagctttgctcacaatgggaacaacaacaataacggcaatggttacacctacacagcgggggaagcctcagtaccttccccagatgggggtcctgagctgcagcctactttcgacccagctcccgccccaccacctgggacaccccttctctgggcccagttcgagcgctctccaggaggtggatctgcagcaccagtatcctcttcctgctcttcttcggcatcctcatctgcctcgtcgtcctctgtggtctttcccgggggtggcgccagcagcacaccctccaatgccaatctggggctgctggtgcaccgtcgactgcacccgggcaccagctgcccgcgcctgtctccgcccttgcacatggccacgggggcgggagagcaccaccttgctcgccgcgtgcgcagcgacccgggcggtggaggcctggcctacgctgcctatgctaatgggctagggacgcagctccctggcctgccctcgtcggacacttcgggctcctcctcgtcctctagctcctcctccagctcttcctcctcttcctctgggctgaggcgcaaaggcagccgcgactgctctgtgtgcttcgagagtgaagtgatcgccgcgctggtgccctgtggccacaacctcttctgcatggagtgtgccaaccgcatttgtgagaagagcgagcccgagtgtcccgtctgccacacggcggtcactcaggccatccgcattttttcctgaaggcagtgcgcgcgcgcgcactgcagggaaggagggtcctctctcgaccctcattccctagggtctacctgcccagacgcctctggtgcccacctctttccaccccaccctcatcactctcagagatcccagaggagcttggaaagctgtagtatccgctcatttttaaaatgtcatttttaaacaaaggaacttgccaggatctctgcatcaggagtactgtagcctccgaaccacctgaattgcatgctctataaataataggaacggcgacattctagtaacgatagtttttacactgtacttaataggaagcttccaaaagaaaaccccacaagttttccattttcttgaagtagaaaaatgaacagtaattatgaagatgattaataattgtgctatgggatgtgtggactgttttgtgtgtttccctttgtgggtgggttcctacagcgctcgttctagaacacaagtggatcctttttgaatgttcatggaagggccaggagttctgtacagccaggaccctgcagctttattaaagttaaaactgtaacatatctcttatatattaaaaaaaaaaacctttaaaagttttaaagagaaattgcattaatacagattgaagtattttattctttttttgacttgaaaaattatatttcatattgcaaagatgtttacaagtattttaatttaagttcagtgaacttttttgtagctgggttaaatctttttatttttagtatggccttatggcaaagaacactgtattattttaataatcacacgattgtgacggattacaaaccataaaatgtataacgttttgagcagtattctgttgggatggagattttataggttcagacaaatcttctagatctgcttcacccagcatattttctattcagtgatataaagcatattttattctatattattacaaaaaatggaaatgtataaacatgtcaaaaggaacagttgatgctttctaacatttgtataaatagaattcagtgcaaattacagaaattctgttgcaccgctatagttttagtgtttctattttaatacatttgtttaccactcgtttatgtatatgtaggtgacgttacttgagcttaaatgtactttactgagcaaagtttaaaaaaaaacaaagtatattttattttatgataaagggcctttaacctcatggtcaaatactaatattatatttgctgagacaagatttgaaattgtatcaagagttttatttttctgacatttaaagttctacataataaaggtaaacttaagtaatggtgctacttcattttttaagtatttctatataaataaaacattgaagaaaaatcact

SEQ ID NO: 5 - protein, 569 aa, Human
MPSSLFADLERNGSGGGGGGSSGGGETLDDQRALQLALDQLSLLGLDSDEGASLYDSEPRKKSVNMTECVPVPSSEHVAEIVGRQGCKIKALRAKTNTYIKTPVRGEEPVFVVTGRKEDVAMARREIISAAEHFSMIRASRNKNTALNGAVPGPPNLPGQTTIQVRVPYRVVGLVVGPKGATIKRIQQQTHTYIVTPSRDKEPVFEVTGMPENVDRAREEIEAHIALRTGGIIELTDENDFHANGTDVGFDLHHGSGGSGPGSLWSKPTPSITPTPGRKPFSSYRNDSSSSLGSASTDSYFGGGTSSSAAATQRLADYSPPSPALSFAHNGNNNNNGNGYTYTAGGEASVPSPDGCPELQPTFDPAPAPPPGAPLIWAQFERSPGGGPAAPVSSSCSSSASSSASSSSVVFPGGGASAPSNANLGLLVHRRLHPGTSCPRLSPPLHMAPGAGEHHLARRVRSDPGGGGLAYAAYANGLGAQLPGLQPSDTSGSSSSSSSSSSSSSSSSGLRRKGSRDCSVCFESEVIAALVPCGHNLFCMECANRICEKSEPECPVCHTAVTQAIRIFS

SEQ ID NO: 6 - protein, 576 aa, Mouse
MPSSLFADLERNGSGGGGGGGGGGGGGGSGGGETLDDQRALQLALDQLSLLGLDSDEGASLYDSEPRKKSVNMTECVPVPSSEHVAEIVGRQGCKIKALRAKTNTYIKTPVRGEEPVFVVTGRKEDVAMARREIISAAEHFSMIRASRNKNTALNGAVPGPPNLPGQTTIQVRVPYRVVGLVVGPKGATIKRIQQQTHTYIVTPSRDKEPVFEVTGMPENVDRAREEIEAHIALRTGGIIELTDENDFHANGTDVGFDLHHGSGGSGPGSLWSKPTPSITPTPGRKPFSSYRNDSSSSLGSASTDSYFGGGTSGSAAATSRLADYSPPSPALSFAHNGNNNNNGNGYTYTAGEASVPSPDGGPELQPTFDPAPAPPPGTPLLWAQFERSPGGGSAAPVSSSCSSSASSSASSSSVVFPGGGASSTPSNANLGLLVHRRLHPGTSCPRLSPPLHMATGAGEHHLARRVRSDPGGGGLAYAAYANGLGTQLPGLPSSDTSGSSSSSSSSSSSSSSSSGLRRKGSRDCSVCFESEVIAALVPCGHNLFCMECANRICEKSEPECPVCHTAVTQAIRIFS

SEQ ID NO: 7 - DNA, 30 bp, Artificial Sequence
  MEX3B primer Fw1
cgtcgtcctctgtggtctttcccgggggtg

SEQ ID NO: 8 - DNA, 30 bp, Artificial Sequence
  MEX3B primer Rv1
tcaggaaaaaatgcggatggcctgagtgac

SEQ ID NO: 9 - DNA, 20 bp, Artificial Sequence
  Mouse GAPDH primer Fw1
agagacagccgcatcttctt

SEQ ID NO: 10 - DNA, 20 bp, Artificial Sequence
  Mouse GAPDH primer Rv1
gacaagcttcccattctcgg

SEQ ID NO: 11 - DNA, 25 bp, Artificial Sequence
  Mouse IL-6 primer Fw1
gctaccaaactggatataatcagga

SEQ ID NO: 12 - DNA, 24 bp, Artificial Sequence
  Mouse IL-6 primer Rv1
ccaggtagctatggtactccagaa

SEQ ID NO: 13 - DNA, 20 bp, Artificial Sequence
  Mouse CXCL5 primer Fw1
cagaaggaggtctgtctgga

SEQ ID NO: 14 - DNA, 20 bp, Artificial Sequence
  Mouse CXCL5 primer Rv1
tgcattccgcttagctttct

SEQ ID NO: 15 - DNA, 4368 bp, Human
tcaagaggcggggaggagaggaggaaaaagcgctgagtgagggcgggcgggcgggcgggagggagggagtggaggagccggggaggggctccttaaagaaacgcttctgtcgctcgcctgctcgcttttcgctcggcattgcggccagccagccgggcactcggggggcacgcgcggccaccgctagagctctgcccccaccccacccgccagcaggtctggggtggggacccaggtgggggctcctgcagccactgcccggtgcggaccgcacggagcgacccactcctcccagcaccgaggaagaagcaacggagccctcagcaggcgaccggcctccccgcccctgaccacccgcttcccggctgcctttgtggccgcagcttctcgccgccgagccgagggccggcgggggcgcggcgcgcacggccgagcgatgcccagctcgctgttcgcagacctggagcgcaacggcagcggcggcggcggcggcggcagcagcggagggggagagaccctggatgaccaaagagccctgcagctcgcgctcgaccagctctccctgctggggctggacagtgacgagggcgcctctctgtacgacagcgagccgcgcaagaagagcgtgaacatgaccgagtgcgtgccagtacccagttctgagcatgtcgccgagatcgtggggcggcaaggtaggtcgaggagggatggggaggtgggtgggggtggtgtagggtctcaggccactgcctcgaggggaaggcgtgttcagtatcgggatccgcggcgtggggtgccttggggagagaggaagagccgcgcgatgggccggcgccccagacaaagaaagtgcaggcaggctgtctcccggagccgcgccgctgccctggcgggatgcactttcttctgctaaaatcactgccttctcccctaacgccccccaaccagcccacctccagaaagacaatttaaatgtaagatgcttgggggagggggcctttgatcagtcctttgggaggaggaaggaggaggagtgagcataggatgggaggaggattctggatttctgcaaagcggaatggagcccagaggaggaacaatgggtcccgggactcacaccccaccccctacccccagtcgaccagcgctgaggcatcgcgacttcagctgccttccccgagccccttccccgtgtcttcagagctgacggcgcgcccagctggatcccagcggcatctccccagatgacttttctgggattctcgggtttggttcgggacgactgcagtcactgggggagggccaggcagccaatgggctgttcctcgagcgcctcgcgggtgggatccgctgcccagcccgtggcgcggcccgaggtcagtgagggagacgccccctttccgcccatctcttgtcctgccgtctcgctgtcctggacgcgggctgtccccggtccccgcggttaccccaggataatgggcgtgtctgtctctctctcccactccctcctccgcaccctggttcgtaggttgtaaaatcaaagcgctgcgggcgaagaccaatacttacatcaagaccccagttcgcggggaggagcctgtctttgttgtgacgggcaggaaggaggatgtggccatggctcggagggagatcatctctgctgccgagcacttctccatgatccgcgcctcccggaataagaacacggcactcaacggcgcggtgcctgggccgcccaacctgcccgggcagaccaccatccaagtgcgggtaccctaccgcgtggtggggctcgtggtggggcccaaaggcgccacaatcaagcgcatccagcagcagacgcacacgtacatcgtgacgcccagccgggataaggagccggtgttcgaggtgaccggcatgccagagaacgtggatcgcgctcgagaggagattgaggcgcacattgctctgcgtaccggcggcatcattgagctcacagacgagaacgacttccacgccaacggcaccgatgtgggcttcgatctgcatcatgggtccggcgggtccggcccaggcagcctctggagcaagcccacccccagcatcacgcccacccccggccgcaagcctttctctagctaccgcaacgacagctccagctcgcttggcagtgcttccacagactcttatttcggcggcgggaccagcagcagcgcagcggctacccagcgcctggcggactacagcccccctagccccgccctgagctttgcgcacaacggaaacaataacaataacggcaatgggtacacctacacagcggggggagaagcctcagtgccatcccccgacggctgccccgagctgcagcccacttttgacccggctcccgctcccccacctggggcaccacttatctgggcccagttcgagcggtccccgggaggcggacctgcagctccggtatcttcttcctgctcttcttctgcatcttcgtctgcttcttcctcctccgtggtcttccccgggggtggcgccagtgcgccctccaacgccaacctggggctattggtgcaccgccggctgcaccctggcaccagctgcccgcgcctgtctccacccttgcacatggccccgggggcgggagagcaccacctggctcgccgggtgcgcagcgacccgggtggaggaggcctggcctacgccgcttatgccaacgggctgggggcacagctgcctggcttgcagccgtcggacacgtcgggctcctcctcttcgtccagctcctcctccagctcttcatcctcttcctccgggcttcggcgtaaaggcagccgcgactgctccgtgtgcttcgagagcgaagtgattgccgcgctggtgccctgtggccacaacctcttctgcatggagtgcgccaatcgcatctgtgagaagagcgagcccgagtgcccggtctgccacaccgcggtcactcaggccatccgcatcttttcttaaaggcagcgggcgctgctagtgcgcaccgtgctgggggaagggggaacccctccccaccctctttccccagcgctcgcctgcctccctgggtgccccccctctcccttctccttcccggccccaccaacactctgagatccgagaggagcttggaaagctgtagtatccgctcatttttaaaatttaatttttaagtaaaggaatttgccaggatatctgcatcaagagtactgtagcctgggaaacctgaacacctgaaatgcatgctctataaataataggaacggcgacattctagtaatgatagtttttacactgtacttaataggaagcttccaaaagaagaaaaccccacaagttttccattttcttaaagtaggaaaaaatgaacagtaataattatgatgaagatgatagtagtgctatgggatgtgtggactgtttagtgtgttcccctttgtgggtgggttcctatgatacttattatagaacacagtggatcctttttgaatgttcgtggaagggccaggagttcctgtgaaaccaggatactgcagctttattaaagttaaagaaactgtaacatatctcttatatattaaaaacgtttaaaagttttaaagagaaattgcattaatacagattgaagtattttattcttttttgacttgaaaaattatatttcatattgcaaagatgtttacaagtattttaatttaagttcagtgaacttttttgtagctgggttaaatctttttattttagtatggccttatggcaaagaacactgtattattttaataatcacacaattgtgacggaattacaaccataaaatgtgtaatgttttgaacagtattctgttgggatggagattttataggttcagacaaatcttctagatctgcttcacccagcatattttctattcagtgatataaagcatattttattctatattattacaaaaacggaaatgtataaacatgtcaaaaagaactgttgatgctttctaacatttgtataaatagaattcagtgcaagttacaaaaattctgttgcaccactctagttttagtatttctattttaatacatttgtttaccacttgtttatgtatatgtaggtgatgttacttgagcttaaatgtactttactgagcaaagtttaaaaaacaaagtatattttattttatgataaagggcctttaacctcatggtcaaatactaatattatatttgctgagacaagatttgaaattgtatcaagagttttatttttctgacatttaaagttctacataataaaggtaaaacttaagtaatggtgctacttcattttttaagtatttctatataaataaaatattgaagaaaatcttaaaaa

SEQ ID NO: 16 - DNA, 15 bp, Artificial Sequence
  mouseMex3bspecific gapmer
acataaacgagtggt

SEQ ID NO: 17 - DNA, 20 bp, Artificial Sequence
  mouseGAPDH-Fw2
tgtgtccgtcgtggatctga

SEQ ID NO: 18 - DNA, 21 bp, Artificial Sequence
  mouseGAPDH-Rv2
ttgctgttgaagtcgcaggag

SEQ ID NO: 19 - DNA, 21 bp, Artificial Sequence
  mouseTNF-Fw
tcttctcattcctgcttgtgg

SEQ ID NO: 20 - DNA, 20 bp, Artificial Sequence
  mouseTNF-Rv
gaggccatttgggaacttct

SEQ ID NO: 21 - DNA, 20 bp, Artificial Sequence
  mouseG-CSF-Fw
cctggagcaagtgaggaaga

SEQ ID NO: 22 - DNA, 20 bp, Artificial Sequence
  mouseG-CSF-Rv
ggggtgacacagcttgtagg

SEQ ID NO: 23 - DNA, 23 bp, Artificial Sequence
  mouseIL-13-Fw
cctctgacccttaaggagcttat

SEQ ID NO: 24 - DNA, 18 bp, Artificial Sequence
  mouseIL-13-Rv
cgttgcacaggggagtct

SEQ ID NO: 25 - DNA, 26 bp, Artificial Sequence
  mouseCXCL2-Fw
aaaatcatccaaaagatactgaacaa

SEQ ID NO: 26 - DNA, 20 bp, Artificial Sequence
  mouseCXCL2-Rv
ctttggttcttccgttgagg

SEQ ID NO: 27 - DNA, 20 bp, Artificial Sequence
  mouseCXCL1-Fw
agactccagccacactccaa

SEQ ID NO: 28 - DNA, 18 bp, Artificial Sequence
  mouseCXCL1-Rv
tgacagcgcagctcattg